European Patent Application EP 4 624 576 A1, published October 1, 2025. Title: A nucleic acid aptamer. Applicant: Xenolis Pte. Ltd. Application JP. The sequence listing filed with the application follows.

SEQUENCE LISTING (214 sequences)

SEQ ID NO: 1 - DNA, 42 bp, synthetic construct
  source 1..42: mol_type = other DNA
  modified_base order(10,31): mod_base = OTHER; note = an unnatural base
cgcggccgangagyaccgaaggtctcrryrnyggaggccgcg

SEQ ID NO: 2 - DNA, 44 bp, synthetic construct
  source 1..44: mol_type = other DNA
  modified_base order(10,22,33): mod_base = OTHER; note = an unnatural base
cgtgaccgangagyacctaacnggtctcrryrnyggaggtcacg

SEQ ID NO: 3 - DNA, 42 bp, synthetic construct
  source 1..42: mol_type = other DNA
  modified_base order(10,31): mod_base = OTHER; note = an unnatural base
cgcggccgangagcaccgaaggtctcaacgntggaggccgcg

SEQ ID NO: 4 - DNA, 44 bp, synthetic construct
  source 1..44: mol_type = other DNA
  modified_base order(10,22,33): mod_base = OTHER; note = an unnatural base
cgtgaccgangagcacctaacnggtctcaacgntggaggtcacg

SEQ ID NO: 5 - DNA, 51 bp, synthetic construct
  source 1..51: mol_type = other DNA
  modified_base order(10,31): mod_base = OTHER; note = an unnatural base
cgcggccgangagyaccgaaggtctcrryrnyggaggccgcgcgcgtagcg

SEQ ID NO: 6 - DNA, 53 bp, synthetic construct
  source 1..53: mol_type = other DNA
  modified_base order(10,22,33): mod_base = OTHER; note = an unnatural base
cgtgaccgangagyacctaacnggtctcrryrnyggaggtcacgcgcgtagcg

SEQ ID NO: 7 - DNA, 51 bp, synthetic construct
  source 1..51: mol_type = other DNA
  modified_base order(10,31): mod_base = OTHER; note = an unnatural base
cgcggccgangagcaccgaaggtctcaacgntggaggccgcgcgcgtagcg

SEQ ID NO: 8 - DNA, 53 bp, synthetic construct
  source 1..53: mol_type = other DNA
  modified_base order(10,22,33): mod_base = OTHER; note = an unnatural base
cgtgaccgangagcacctaacnggtctcaacgntggaggtcacgcgcgtagcg

SEQ ID NO: 9 - DNA, 44 bp, synthetic construct
  source 1..44: mol_type = other DNA
  modified_base order(10,22,33): mod_base = OTHER; note = an unnatural base
cgtgaccgangagtacctaacnggtctcaacgntggaggtcacg

SEQ ID NO: 10 - DNA, 44 bp, synthetic construct
  source 1..44: mol_type = other DNA
  modified_base order(10,22,33): mod_base = OTHER; note = an unnatural base
cgtgaccgangagcacctaacnggtctcgacgntggaggtcacg

SEQ ID NO: 11 - DNA, 44 bp, synthetic construct
  source 1..44: mol_type = other DNA
  modified_base order(10,22,33): mod_base = OTHER; note = an unnatural base
cgtgaccgangagcacctaacnggtctcagcgntggaggtcacg

SEQ ID NO: 12 - DNA, 44 bp, synthetic construct
  source 1..44: mol_type = other DNA
  modified_base order(10,22,33): mod_base = OTHER; note = an unnatural base
cgtgaccgangagcacctaacnggtctcaatgntggaggtcacg

SEQ ID NO: 13 - DNA, 44 bp, synthetic construct
  source 1..44: mol_type = other DNA
  modified_base order(10,22,33): mod_base = OTHER; note = an unnatural base
cgtgaccgangagcacctaacnggtctcaacantggaggtcacg

SEQ ID NO: 14 - DNA, 44 bp, synthetic construct
  source 1..44: mol_type = other DNA
  modified_base order(10,22,33): mod_base = OTHER; note = an unnatural base
cgtgaccgangagcacctaacnggtctcaacgncggaggtcacg

SEQ ID NO: 15 - DNA, 48 bp, synthetic construct
  source 1..48: mol_type = other DNA
  modified_base order(28,39): mod_base = OTHER; note = an unnatural base
cccgcccgggtccgcgaagcggtaggtnygggctaggcngyyggcggg

SEQ ID NO: 16 - DNA, 49 bp, synthetic construct
  source 1..49: mol_type = other DNA
  modified_base order(18,29,40): mod_base = OTHER; note = an unnatural base
tcctctcgggtcatttantaatgtaggtnygggctaggcngyyagtgga

SEQ ID NO: 17 - DNA, 48 bp, synthetic construct
  source 1..48: mol_type = other DNA
  modified_base order(28,39): mod_base = OTHER; note = an unnatural base
cccgcccgggtccgcgaagcggtaggtntgggctaggcngctggcggg

SEQ ID NO: 18 - DNA, 49 bp, synthetic construct
  source 1..49: mol_type = other DNA
  modified_base order(18,29,40): mod_base = OTHER; note = an unnatural base
tcctctcgggtcatttantaatgtaggtntgggctaggcngctagtgga

SEQ ID NO: 19 - DNA, 57 bp, synthetic construct
  source 1..57: mol_type = other DNA
  modified_base order(28,39): mod_base = OTHER; note = an unnatural base
cccgcccgggtccgcgaagcggtaggtnygggctaggcngyyggcgggcgcgtagcg

SEQ ID NO: 20 - DNA, 58 bp, synthetic construct
  source 1..58: mol_type = other DNA
  modified_base order(18,29,40): mod_base = OTHER; note = an unnatural base
tcctctcgggtcatttantaatgtaggtnygggctaggcngyyagtggacgcgtagcg

SEQ ID NO: 21 - DNA, 57 bp, synthetic construct
  source 1..57: mol_type = other DNA
  modified_base order(28,39): mod_base = OTHER; note = an unnatural base
cccgcccgggtccgcgaagcggtaggtntgggctaggcngctggcgggcgcgtagcg

SEQ ID NO: 22 - DNA, 58 bp, synthetic construct
  source 1..58: mol_type = other DNA
  modified_base order(18,29,40): mod_base = OTHER; note = an unnatural base
tcctctcgggtcatttantaatgtaggtntgggctaggcngctagtggacgcgtagcg

SEQ ID NO: 23 - DNA, 49 bp, synthetic construct
  source 1..49: mol_type = other DNA
  modified_base order(18,29,40): mod_base = OTHER; note = an unnatural base
tcctctcgggtcatttantaatgtaggtncgggctaggcngctagtgga

SEQ ID NO: 24 - DNA, 49 bp, synthetic construct
  source 1..49: mol_type = other DNA
  modified_base order(18,29,40): mod_base = OTHER; note = an unnatural base
tcctctcgggtcatttantaatgtaggtntgggctaggcngttagtgga

SEQ ID NO: 25 - DNA, 49 bp, synthetic construct
  source 1..49: mol_type = other DNA
  modified_base order(18,29,40): mod_base = OTHER; note = an unnatural base
tcctctcgggtcatttantaatgtaggtntgggctaggcngccagtgga

SEQ ID NO: 26 - DNA, 47 bp, synthetic construct
  source 1..47: mol_type = other DNA
  modified_base order(24,33): mod_base = OTHER; note = an unnatural base
cggtaaactgcgtccgaaggggcntgcagtgancccgaatgggtccg

SEQ ID NO: 27 - DNA, 39 bp, synthetic construct
  source 1..39: mol_type = other DNA
  modified_base order(19,25): mod_base = OTHER; note = an unnatural base
ccccagacggrctggtgynctcggnatgrccgtctgggg

SEQ ID NO: 28 - DNA, 31 bp, synthetic construct
  source 1..31: mol_type = other DNA
  modified_base order(15,21): mod_base = OTHER; note = an unnatural base
caatggrctggtgynctcggnatgrccattg

SEQ ID NO: 29 - DNA, 39 bp, synthetic construct
  source 1..39: mol_type = other DNA
  modified_base order(19,25): mod_base = OTHER; note = an unnatural base
ccccagacggactggtgtnctcggnatggccgtctgggg

SEQ ID NO: 30 - DNA, 31 bp, synthetic construct
  source 1..31: mol_type = other DNA
  modified_base order(15,21): mod_base = OTHER; note = an unnatural base
caatggactggtgtnctcggnatggccattg

SEQ ID NO: 31 - DNA, 48 bp, synthetic construct
  source 1..48: mol_type = other DNA
  modified_base order(19,25): mod_base = OTHER; note = an unnatural base
ccccagacggrctggtgynctcggnatgrccgtctggggcgcgaagcg

SEQ ID NO: 32 - DNA, 40 bp, synthetic construct
  source 1..40: mol_type = other DNA
  modified_base order(15,21): mod_base = OTHER; note = an unnatural base
caatggrctggtgynctcggnatgrccattgcgcgaagcg

SEQ ID NO: 33 - DNA, 48 bp, synthetic construct
  source 1..48: mol_type = other DNA
  modified_base order(19,25): mod_base = OTHER; note = an unnatural base
ccccagacggactggtgtnctcggnatggccgtctggggcgcgaagcg

SEQ ID NO: 34 - DNA, 40 bp, synthetic construct
  source 1..40: mol_type = other DNA
  modified_base order(15,21): mod_base = OTHER; note = an unnatural base
caatggactggtgtnctcggnatggccattgcgcgaagcg

SEQ ID NO: 35 - DNA, 31 bp, synthetic construct
  source 1..31: mol_type = other DNA
  modified_base order(15,21): mod_base = OTHER; note = an unnatural base
caatgggctggtgtnctcggnatggccattg

SEQ ID NO: 36 - DNA, 31 bp, synthetic construct
  source 1..31: mol_type = other DNA
  modified_base order(15,21): mod_base = OTHER; note = an unnatural base
caatggactggtgcnctcggnatggccattg

SEQ ID NO: 37 - DNA, 31 bp, synthetic construct
  source 1..31: mol_type = other DNA
  modified_base order(15,21): mod_base = OTHER; note = an unnatural base
caatggactggtgtnctcggnatgaccattg

SEQ ID NO: 38 - DNA, 50 bp, synthetic construct
  source 1..50: mol_type = other DNA
  modified_base order(15,23): mod_base = OTHER; note = an unnatural base
ccgcttgtcatcyanccyggccnygtggyryygtarcggytgacaagcgg

SEQ ID NO: 39 - DNA, 30 bp, synthetic construct
  source 1..30: mol_type = other DNA
  modified_base order(11,19): mod_base = OTHER; note = an unnatural base
tcyanccyggccnygtggyryygtarcggy

SEQ ID NO: 40 - DNA, 50 bp, synthetic construct
  source 1..50: mol_type = other DNA
  modified_base order(15,23): mod_base = OTHER; note = an unnatural base
ccgcttgtcatctancctggccntgtggtactgtaacggctgacaagcgg

SEQ ID NO: 41 - DNA, 42 bp, synthetic construct
  source 1..42: mol_type = other DNA
  modified_base order(11,19): mod_base = OTHER; note = an unnatural base
ttgtcatctancctggccntgtggtactgtaacggctgacaa

SEQ ID NO: 42 - DNA, 59 bp, synthetic construct
  source 1..59: mol_type = other DNA
  modified_base order(15,23): mod_base = OTHER; note = an unnatural base
ccgcttgtcatcyanccyggccnygtggyryygtarcggytgacaagcggcgcgtagcg

SEQ ID NO: 43 - DNA, 51 bp, synthetic construct
  source 1..51: mol_type = other DNA
  modified_base order(11,19): mod_base = OTHER; note = an unnatural base
ttgtcatcyanccyggccnygtggyryygtarcggytgacaacgcgtagcg

SEQ ID NO: 44 - DNA, 59 bp, synthetic construct
  source 1..59: mol_type = other DNA
  modified_base order(15,23): mod_base = OTHER; note = an unnatural base
ccgcttgtcatctancctggccntgtggtactgtaacggctgacaagcggcgcgtagcg

SEQ ID NO: 45 - DNA, 51 bp, synthetic construct
  source 1..51: mol_type = other DNA
  modified_base order(11,19): mod_base = OTHER; note = an unnatural base
ttgtcatctancctggccntgtggtactgtaacggctgacaacgcgtagcg

SEQ ID NO: 46 - DNA, 42 bp, synthetic construct
  source 1..42: mol_type = other DNA
  modified_base order(11,19): mod_base = OTHER; note = an unnatural base
ttgtcatccancctggccntgtggtactgtaacggctgacaa

SEQ ID NO: 47 - DNA, 42 bp, synthetic construct
  source 1..42: mol_type = other DNA
  modified_base order(11,19): mod_base = OTHER; note = an unnatural base
ttgtcatctancccggccntgtggtactgtaacggctgacaa

SEQ ID NO: 48 - DNA, 42 bp, synthetic construct
  source 1..42: mol_type = other DNA
  modified_base order(11,19): mod_base = OTHER; note = an unnatural base
ttgtcatctancctggccncgtggtactgtaacggctgacaa

SEQ ID NO: 49 - DNA, 42 bp, synthetic construct
  source 1..42: mol_type = other DNA
  modified_base order(11,19): mod_base = OTHER; note = an unnatural base
ttgtcatctancctggccntgtggcactgtaacggctgacaa

SEQ ID NO: 50 - DNA, 42 bp, synthetic construct
  source 1..42: mol_type = other DNA
  modified_base order(11,19): mod_base = OTHER; note = an unnatural base
ttgtcatctancctggccntgtggtgctgtaacggctgacaa

SEQ ID NO: 51 - DNA, 42 bp, synthetic construct
  source 1..42: mol_type = other DNA
  modified_base order(11,19): mod_base = OTHER; note = an unnatural base
ttgtcatctancctggccntgtggtattgtaacggctgacaa

SEQ ID NO: 52 - DNA, 42 bp, synthetic construct
  source 1..42: mol_type = other DNA
  modified_base order(11,19): mod_base = OTHER; note = an unnatural base
ttgtcatctancctggccntgtggtaccgtaacggctgacaa

SEQ ID NO: 53 - DNA, 42 bp, synthetic construct
  source 1..42: mol_type = other DNA
  modified_base order(11,19): mod_base = OTHER; note = an unnatural base
ttgtcatctancctggccntgtggtactgtagcggctgacaa

SEQ ID NO: 54 - DNA, 42 bp, synthetic construct
  source 1..42: mol_type = other DNA
  modified_base order(11,19): mod_base = OTHER; note = an unnatural base
ttgtcatctancctggccntgtggtactgtaacggttgacaa

SEQ ID NO: 55 - DNA, 52 bp, synthetic construct
  source 1..52: mol_type = other DNA
  modified_base order(22,28,34): mod_base = OTHER; note = an unnatural base
ctccgcagtctgtggtgggacngggctnatgtangggatctgacaagcggag

SEQ ID NO: 56 - DNA, 31 bp, synthetic construct
  source 1..31: mol_type = other DNA
  modified_base order(12,18,24): mod_base = OTHER; note = an unnatural base
tgtggtgggacngggctnatgtangggatct

SEQ ID NO: 57 - DNA, 49 bp, synthetic construct
  source 1..49: mol_type = other DNA
  modified_base order(21,27,33): mod_base = OTHER; note = an unnatural base
ctccgcgtctgtggtgggacngggctnatgtangggatctgacgcggag

SEQ ID NO: 58 - DNA, 49 bp, synthetic construct
  source 1..49: mol_type = other DNA
  modified_base order(27,33): mod_base = OTHER; note = an unnatural base
ctccgcgtctgtggtgggactgggctnatgtangggatctgacgcggag

SEQ ID NO: 59 - DNA, 31 bp, synthetic construct
  source 1..31: mol_type = other DNA
  modified_base order(18,24): mod_base = OTHER; note = an unnatural base
tgtggtgggactgggctnatgtangggatct

SEQ ID NO: 60 - DNA, 49 bp, synthetic construct
  source 1..49: mol_type = other DNA
  modified_base order(21,33): mod_base = OTHER; note = an unnatural base
ctccgcgtctgtggtgggacngggctaatgtangggatctgacgcggag

SEQ ID NO: 61 - DNA, 31 bp, synthetic construct
  source 1..31: mol_type = other DNA
  modified_base order(12,24): mod_base = OTHER; note = an unnatural base
tgtggtgggacngggctaatgtangggatct

SEQ ID NO: 62 - DNA, 54 bp, synthetic construct
  source 1..54: mol_type = other DNA
  modified_base order(24,37): mod_base = OTHER; note = an unnatural base
gtcctcacgccgtcataattgttnttttgatccttgnagtggggacgtgaggac

SEQ ID NO: 63 - DNA, 36 bp, synthetic construct
  source 1..36: mol_type = other DNA
  modified_base order(15,28): mod_base = OTHER; note = an unnatural base
ccgtcataattgttnttttgatccttgnagtgggga

SEQ ID NO: 64 - DNA, 54 bp, synthetic construct
  source 1..54: mol_type = other DNA
  modified_base order(17,24,37): mod_base = OTHER; note = an unnatural base
gtcctcacgccgtcatnattgttnttttgatccttgnagtggggacgtgaggac

SEQ ID NO: 65 - DNA, 36 bp, synthetic construct
  source 1..36: mol_type = other DNA
  modified_base order(8,15,28): mod_base = OTHER; note = an unnatural base
ccgtcatnattgttnttttgatccttgnagtgggga

SEQ ID NO: 66 - DNA, 54 bp, synthetic construct
  source 1..54: mol_type = other DNA
  modified_base order(18,24,37): mod_base = OTHER; note = an unnatural base
gtcctcacgccgtcatanttgttnttttgatccttgnagtggggacgtgaggac

SEQ ID NO: 67 - DNA, 36 bp, synthetic construct
  source 1..36: mol_type = other DNA
  modified_base order(9,15,28): mod_base = OTHER; note = an unnatural base
ccgtcatanttgttnttttgatccttgnagtgggga

SEQ ID NO: 68 - DNA, 54 bp, synthetic construct; identical to SEQ ID NO: 64
  source 1..54: mol_type = other DNA
  modified_base order(17,24,37): mod_base = OTHER; note = an unnatural base

SEQ ID NO: 69 - DNA, 36 bp, synthetic construct; identical to SEQ ID NO: 65
  source 1..36: mol_type = other DNA
  modified_base order(8,15,28): mod_base = OTHER; note = an unnatural base

SEQ ID NO: 70 - DNA, 54 bp, synthetic construct; identical to SEQ ID NO: 66
  source 1..54: mol_type = other DNA
  modified_base order(18,24,37): mod_base = OTHER; note = an unnatural base

SEQ ID NO: 71 - DNA, 36 bp, synthetic construct; identical to SEQ ID NO: 67
  source 1..36: mol_type = other DNA
  modified_base order(9,15,28): mod_base = OTHER; note = an unnatural base

SEQ ID NO: 72 - DNA, 54 bp, synthetic construct
  source 1..54: mol_type = other DNA
  modified_base order(17,18,24,37): mod_base = OTHER; note = an unnatural base
gtcctcacgccgtcatnnttgttnttttgatccttgnagtggggacgtgaggac

SEQ ID NO: 73 - DNA, 36 bp, synthetic construct
  source 1..36: mol_type = other DNA
  modified_base order(8,9,15,28): mod_base = OTHER; note = an unnatural base
ccgtcatnnttgttnttttgatccttgnagtgggga

SEQ ID NO: 74 - DNA, 51 bp, synthetic construct
  source 1..51: mol_type = other DNA
  modified_base order(9,20,32): mod_base = OTHER; note = an unnatural base
gctgcttcngccatgacccntttcagccggcntggtcatgtgacaagcagc

SEQ ID NO: 75 - DNA, 15 bp, synthetic construct
  source 1..15: mol_type = other DNA
  modified_base order(2,14): mod_base = OTHER; note = an unnatural base
cntttcagccggcnt

SEQ ID NO: 76 - DNA, 51 bp, synthetic construct
  source 1..51: mol_type = other DNA
  modified_base order(20,32): mod_base = OTHER; note = an unnatural base
gctgcttcagccatgacccntttcagccggcntggtcatgtgacaagcagc

SEQ ID NO: 77 - DNA, 50 bp, synthetic construct
  source 1..50: mol_type = other DNA
  modified_base order(9,20,31): mod_base = OTHER; note = an unnatural base
gctgcttcngccatgacccnttcagccggcntggtcatgtgacaagcagc

SEQ ID NO: 78 - DNA, 14 bp, synthetic construct
  source 1..14: mol_type = other DNA
  modified_base order(2,13): mod_base = OTHER; note = an unnatural base
cnttcagccggcnt

SEQ ID NO: 79 - DNA, 39 bp, synthetic construct
  source 1..39: mol_type = other DNA
  modified_base order(14,26): mod_base = OTHER; note = an unnatural base
cgctgcatgacccntttcagccggcntggtcatgcagcg

SEQ ID NO: 80 - DNA, 38 bp, synthetic construct
  source 1..38: mol_type = other DNA
  modified_base order(14,25): mod_base = OTHER; note = an unnatural base
cgctgcatgacccnttcagccggcntggtcatgcagcg

SEQ ID NO: 81 - DNA, 48 bp, synthetic construct
  source 1..48: mol_type = other DNA
  modified_base order(16,22): mod_base = OTHER; note = an unnatural base
gtcacgcgctgtggtngttttnttgggggggtggttaaggcgcgtgac

SEQ ID NO: 82 - DNA, 28 bp, synthetic construct
  source 1..28: mol_type = other DNA
  modified_base order(6,12): mod_base = OTHER; note = an unnatural base
gtggtngttttnttgggggggtggttaa

SEQ ID NO: 83 - DNA, 43 bp, synthetic construct
  source 1..43: mol_type = other DNA
  modified_base order(10,16,28): mod_base = OTHER; note = an unnatural base
gcacgctttnacttantggctgggtggnctgggtaaagcgtgc

SEQ ID NO: 84 - DNA, 25 bp, synthetic construct
  source 1..25: mol_type = other DNA
  modified_base order(1,7,19): mod_base = OTHER; note = an unnatural base
nacttantggctgggtggnctgggt

SEQ ID NO: 85 - DNA, 53 bp, synthetic construct
  source 1..53: mol_type = other DNA
  modified_base order(26,41): mod_base = OTHER; note = an unnatural base
gctgtcacgcagcatggaacctttantggctaggggtgggnggaggtgacagc

SEQ ID NO: 86 - DNA, 37 bp, synthetic construct
  source 1..37: mol_type = other DNA
  modified_base order(18,33): mod_base = OTHER; note = an unnatural base
gcagcatggaacctttantggctaggggtgggnggag

SEQ ID NO: 87 - DNA, 51 bp, synthetic construct
  source 1..51: mol_type = other DNA
  modified_base order(16,24,35): mod_base = OTHER; note = an unnatural base
gcgttgcgtgaagttngggtgggnatgtgatgggnggtagatagacaacgc

SEQ ID NO: 88 - DNA, 39 bp, synthetic construct
  source 1..39: mol_type = other DNA
  modified_base order(10,18,29): mod_base = OTHER; note = an unnatural base
cgtgaagttngggtgggnatgtgatgggnggtagataga

SEQ ID NO: 89 - DNA, 51 bp, synthetic construct
  source 1..51: mol_type = other DNA
  modified_base order(17,24,36,39): mod_base = OTHER; note = an unnatural base
gctgatctcggaagganggtgggntctgggttgggnggngcgtagatcagc

SEQ ID NO: 90 - DNA, 35 bp, synthetic construct
  source 1..35: mol_type = other DNA
  modified_base order(9,16,28,31): mod_base = OTHER; note = an unnatural base
cggaagganggtgggntctgggttgggnggngcgt

SEQ ID NO: 91 - DNA, 46 bp, synthetic construct
  source 1..46: mol_type = other DNA
  modified_base order(29,38): mod_base = OTHER; note = an unnatural base
gcacgaggcagggttgggagggtaagganggtgggtgncctcgtgc

SEQ ID NO: 92 - DNA, 25 bp, synthetic construct
  source 1..25: mol_type = other DNA
  modified_base 19: mod_base = OTHER; note = an unnatural base
gggttgggagggtaagganggtggg

SEQ ID NO: 93 - DNA, 43 bp, synthetic construct
  source 1..43: mol_type = other DNA
  modified_base order(13,20,25,34): mod_base = OTHER; note = an unnatural base
gcacgtggggtcnccgatgnccatnaccacaggnaccacgtgc

SEQ ID NO: 94 - DNA, 23 bp, synthetic construct
  source 1..23: mol_type = other DNA
  modified_base order(2,9,14,23): mod_base = OTHER; note = an unnatural base
cnccgatgnccatnaccacaggn

SEQ ID NO: 95 - DNA, 57 bp, synthetic construct
  source 1..57: mol_type = other DNA
  modified_base order(17,33,38): mod_base = OTHER; note = an unnatural base
gctccgcgccgtacacnagtccgctagacatgncagtnacgagtggacaagcggagc

SEQ ID NO: 96 - DNA, 26 bp, synthetic construct
  source 1..26: mol_type = other DNA
  modified_base order(1,17,22): mod_base = OTHER; note = an unnatural base
nagtccgctagacatgncagtnacga

SEQ ID NO: 97 - DNA, 45 bp, synthetic construct
  source 1..45: mol_type = other DNA
  modified_base order(17,26): mod_base = OTHER; note = an unnatural base
ggagatgctaactcaanccggtggcnaggcgagttgaacatctcc

SEQ ID NO: 98 - DNA, 16 bp, synthetic construct
  source 1..16: mol_type = other DNA
  modified_base order(3,12): mod_base = OTHER; note = an unnatural base
aanccggtggcnaggc

SEQ ID NO: 99 - DNA, 45 bp, synthetic construct
  source 1..45: mol_type = other DNA
  modified_base order(17,26): mod_base = OTHER; note = an unnatural base
gactccgcttgaacaanccggtgggnaggcgtgacaagcggagtc

SEQ ID NO: 100 - DNA, 16 bp, synthetic construct
  source 1..16: mol_type = other DNA
  modified_base order(3,12): mod_base = OTHER; note = an unnatural base
aanccggtgggnaggc

SEQ ID NO: 101 - DNA, 45 bp, synthetic construct
  source 1..45: mol_type = other DNA
  modified_base order(17,26,37): mod_base = OTHER; note = an unnatural base
ggagatgctaactcaanccggtggcnaggcgagttgnacatctcc

SEQ ID NO: 102 - DNA, 42 bp, synthetic construct
  source 1..42: mol_type = other DNA
  modified_base order(16,25): mod_base = OTHER; note = an unnatural base
gactccgcttgacaanccggtgggnaggcgtcaagcggagtc

SEQ ID NO: 103 - DNA, 50 bp, synthetic construct
  source 1..50: mol_type = other DNA
  modified_base order(17,23,30): mod_base = OTHER; note = an unnatural base
gttcacgagagtgtgcnccatancacgggnaggtgacatatatcgtgaac

SEQ ID NO: 104 - DNA, 21 bp, synthetic construct
  source 1..21: mol_type = other DNA
  modified_base order(3,9,16): mod_base = OTHER; note = an unnatural base
gcnccatancacgggnaggtg

SEQ ID NO: 105 - DNA, 10 bp, synthetic construct
  source 1..10: mol_type = other DNA
ctccgcagtc

SEQ ID NO: 106 - DNA, 11 bp, synthetic construct
  source 1..11: mol_type = other DNA
gacaagcggag

SEQ ID NO: 107-110 - skipped (4 entries)

SEQ ID NO: 111 - DNA, 18 bp, synthetic construct
  source 1..18: mol_type = other DNA
  modified_base 9: mod_base = OTHER; note = an unnatural base
gctgcttcngccatgacc

SEQ ID NO: 112 - DNA, 18 bp, synthetic construct
  source 1..18: mol_type = other DNA
ggtcatgtgacaagcagc

SEQ ID NO: 113 - DNA, 18 bp, synthetic construct
  source 1..18: mol_type = other DNA
gctgcttcagccatgacc

SEQ ID NO: 114 - skipped

SEQ ID NO: 115 - DNA, 12 bp, synthetic construct
  source 1..12: mol_type = other DNA
cgctgcatgacc

SEQ ID NO: 116 - DNA, 12 bp, synthetic construct
  source 1..12: mol_type = other DNA
ggtcatgcagcg

SEQ ID NO: 117 - DNA, 10 bp, synthetic construct
  source 1..10: mol_type = other DNA
gtcacgcgct

SEQ ID NO: 118 - DNA, 10 bp, synthetic construct
  source 1..10: mol_type = other DNA
ggcgcgtgac

SEQ ID NO: 119-126 - skipped (8 entries)

SEQ ID NO: 127 - DNA, 10 bp, synthetic construct
  source 1..10: mol_type = other DNA
gcacgaggca

SEQ ID NO: 128 - DNA, 11 bp, synthetic construct
  source 1..11: mol_type = other DNA
  modified_base 3: mod_base = OTHER; note = an unnatural base
tgncctcgtgc

SEQ ID NO: 129 - DNA, 11 bp, synthetic construct
  source 1..11: mol_type = other DNA
gcacgtggggt

SEQ ID NO: 130 - skipped

SEQ ID NO: 131 - DNA, 16 bp, synthetic construct
  source 1..16: mol_type = other DNA
gctccgcgccgtacac

SEQ ID NO: 132 - DNA, 15 bp, synthetic construct
  source 1..15: mol_type = other DNA
gtggacaagcggagc

SEQ ID NO: 133 - DNA, 14 bp, synthetic construct
  source 1..14: mol_type = other DNA
ggagatgctaactc

SEQ ID NO: 134 - DNA, 15 bp, synthetic construct
  source 1..15: mol_type = other DNA
gagttgaacatctcc

SEQ ID NO: 135 - DNA, 14 bp, synthetic construct
  source 1..14: mol_type = other DNA
gactccgcttgaac

SEQ ID NO: 136 - DNA, 15 bp, synthetic construct
  source 1..15: mol_type = other DNA
gtgacaagcggagtc

SEQ ID NO: 137 - DNA, 15 bp, synthetic construct
  source 1..15: mol_type = other DNA
  modified_base 7: mod_base = OTHER; note = an unnatural base
gagttgnacatctcc

SEQ ID NO: 138 - DNA, 13 bp, synthetic construct
  source 1..13: mol_type = other DNA
gactccgcttgac

SEQ ID NO: 139 - DNA, 13 bp, synthetic construct
  source 1..13: mol_type = other DNA
gtcaagcggagtc

SEQ ID NO: 140 - DNA, 14 bp, synthetic construct
  source 1..14: mol_type = other DNA
gttcacgagagtgt

SEQ ID NO: 141 - DNA, 15 bp, synthetic construct
  source 1..15: mol_type = other DNA
acatatatcgtgaac

SEQ ID NO: 142 - DNA, 57 bp, synthetic construct
  source 1..57: mol_type = other DNA
  modified_base order(16,22): mod_base = OTHER; note = an unnatural base
gtcacgcgctgtggtngttttnttgggggggtggttaaggcgcgtgaccgcgtagcg

SEQ ID NO: 143 - DNA, 61 bp, synthetic construct
  source 1..61: mol_type = other DNA
  modified_base order(22,33): mod_base = OTHER; note = an unnatural base
ctccttcagcgccaccgtatgnacgctcacagnagttgccgagctgaaggagcgcgtagcg

SEQ ID NO: 144 - DNA, 61 bp, synthetic construct
  source 1..61: mol_type = other DNA
ctccttcagcgccaccgtatgaacgctcacagaagttgccgagctgaaggagcgcgtagcg

SEQ ID NO: 145 - DNA, 54 bp, synthetic construct
  source 1..54: mol_type = other DNA
  modified_base 37: mod_base = OTHER; note = an unnatural base
gtcctcacgccgtcataattgttattttgatccttgnagtggggacgtgaggac

SEQ ID NO: 146 - DNA, 57 bp, synthetic construct; identical to SEQ ID NO: 21
  source 1..57: mol_type = other DNA
  modified_base order(28,39): mod_base = OTHER; note = an unnatural base

SEQ ID NO: 147 - DNA, 63 bp, synthetic construct
  source 1..63: mol_type = other DNA
  modified_base 37: mod_base = OTHER; note = an unnatural base
gtcctcacgccgtcataattgttattttgatccttgnagtggggacgtgaggaccgcgtagcg

SEQ ID NO: 148 - DNA, 63 bp, synthetic construct
  source 1..63: mol_type = other DNA
  modified_base order(24,37): mod_base = OTHER; note = an unnatural base
gtcctcacgccgtcataattgttnttttgatccttgnagtggggacgtgaggaccgcgtagcg

SEQ ID NO: 149 - DNA, 70 bp, synthetic construct
  source 1..70: mol_type = other DNA
  modified_base order(14,27): mod_base = OTHER; note = an unnatural base
ggctggtccggggcccgtantcagacgtatacncatcagggcacatacaagcggaccagcccgcgtagcg

SEQ ID NO: 150 - DNA, 51 bp, synthetic construct
  source 1..51: mol_type = other DNA
  modified_base order(14,27): mod_base = OTHER; note = an unnatural base
ggtccggcccgtantcagacgtatacncatcagggccggacccgcgtagcg

SEQ ID NO: 151 - DNA, 51 bp, synthetic construct
  source 1..51: mol_type = other DNA
ggtccggcccgtaatcagacgtatacacatcagggccggacccgcgtagcg

SEQ ID NO: 152 - DNA, 59 bp, synthetic construct
  source 1..59: mol_type = other DNA
  modified_base order(14,35): mod_base = OTHER; note = an unnatural base
ggctggtccgtacncccaacctttccaatccagcnttagccggaccagcccgcgtagcg

SEQ ID NO: 153 - DNA, 63 bp, synthetic construct
  source 1..63: mol_type = other DNA
  modified_base order(17,21,36): mod_base = OTHER; note = an unnatural base
ggctggtccgccaatcnagcntagtctaaaagaccncccaaccccggaccagcccgcgtagcg

SEQ ID NO: 154 - DNA, 63 bp, synthetic construct
  source 1..63: mol_type = other DNA
  modified_base order(18,35,43): mod_base = OTHER; note = an unnatural base
ggctggtccgtccagcanccaatctccaccaaccncctgccangcggaccagcccgcgtagcg

SEQ ID NO: 155 - DNA, 53 bp, synthetic construct
  source 1..53: mol_type = other DNA
  modified_base 13: mod_base = OTHER; note = an unnatural base
ggctggtccgcgnccaacctccaccaatcaaagccggaccagcccgcgtagcg

SEQ ID NO: 156 - DNA, 57 bp, synthetic construct
  source 1..57: mol_type = other DNA
  modified_base order(18,28): mod_base = OTHER; note = an unnatural base
cggcggagacgtaacgcntatcaaatcnaaacagcttagggtccgccgcgcgtagcg

SEQ ID NO: 157 - DNA, 58 bp, synthetic construct
  source 1..58: mol_type = other DNA
  modified_base order(25,34): mod_base = OTHER; note = an unnatural base
gcggtaagccgcgtccgaaggggcntgcggcgancccgaatgggtccgccgcgtagcg

SEQ ID NO: 158 - DNA, 58 bp, synthetic construct
  source 1..58: mol_type = other DNA
gcggtaagccgcgtccgaaggggcatgcggcgaacccgaatgggtccgccgcgtagcg

SEQ ID NO: 159 - DNA, 45 bp, synthetic construct
  source 1..45: mol_type = other DNA
  modified_base 27: mod_base = OTHER; note = an unnatural base
ggcgccaggggtgtttgtgccgtgagntgtggcgcccgcgtagcg

SEQ ID NO: 160 - DNA, 45 bp, synthetic construct
  source 1..45: mol_type = other DNA
ggcgccaggggtgtttgtgccgtgagatgtggcgcccgcgtagcg

SEQ ID NO: 161 - DNA, 52 bp, synthetic construct
  source 1..52: mol_type = other DNA
ctccgcagtctgtggtgggactgggctaatgtaagggatctgacaagcggag

SEQ ID NO: 162 - DNA, 49 bp, synthetic construct
  source 1..49: mol_type = other DNA
  modified_base order(21,27): mod_base = OTHER; note = an unnatural base
ctccgcgtctgtggtgggacngggctnatgtaagggatctgacgcggag

SEQ ID NO: 163 - DNA, 58 bp, synthetic construct
  source 1..58: mol_type = other DNA
  modified_base order(21,27,33): mod_base = OTHER; note = an unnatural base
ctccgcgtctgtggtgggacngggctnatgtangggatctgacgcggagcgcgtagcg

SEQ ID NO: 164 - DNA, 48 bp, synthetic construct; identical to SEQ ID NO: 17
  source 1..48: mol_type = other DNA
  modified_base order(23,39): mod_base = OTHER; note = an unnatural base

SEQ ID NO: 165 - DNA, 57 bp, synthetic construct; identical to SEQ ID NO: 21
  source 1..57: mol_type = other DNA
  modified_base order(28,39): mod_base = OTHER; note = an unnatural base

SEQ ID NO: 166 - DNA, 54 bp, synthetic construct
  source 1..54: mol_type = other DNA
  modified_base order(13,24,37): mod_base = OTHER; note = an unnatural base
gtcctcacgccgncataattgttnttttgatccttgnagtggggacgtgaggac

SEQ ID NO: 167 - DNA, 54 bp, synthetic construct
  source 1..54: mol_type = other DNA
  modified_base order(24,31,37): mod_base = OTHER; note = an unnatural base
gtcctcacgccgtcataattgttnttttganccttgnagtggggacgtgaggac

SEQ ID NO: 168 - DNA, 54 bp, synthetic construct; identical to SEQ ID NO: 62
  source 1..54: mol_type = other DNA
  modified_base order(24,37): mod_base = OTHER; note = an unnatural base

SEQ ID NO: 169 - DNA, 54 bp, synthetic construct; identical to SEQ ID NO: 64
  source 1..54: mol_type = other DNA
  modified_base order(17,24,37): mod_base = OTHER; note = an unnatural base

SEQ ID NO: 170 - DNA, 54 bp, synthetic construct; identical to SEQ ID NO: 66
  source 1..54: mol_type = other DNA
  modified_base order(18,24,37): mod_base = OTHER; note = an unnatural base

SEQ ID NO: 171 - DNA, 63 bp, synthetic construct; identical to SEQ ID NO: 148
  source 1..63: mol_type = other DNA
  modified_base order(24,37): mod_base = OTHER; note = an unnatural base

SEQ ID NO: 172 - DNA, 63 bp, synthetic construct
  source 1..63: mol_type = other DNA
  modified_base order(18,24,37): mod_base = OTHER; note = an unnatural base
gtcctcacgccgtcatanttgttnttttgatccttgnagtggggacgtgaggaccgcgtagcg

SEQ ID NO: 173 - DNA, 50 bp, synthetic construct
  source 1..50: mol_type = other DNA
  modified_base order(22,31): mod_base = OTHER; note = an unnatural base
gctgtcccgccgcgcagattantggtttganatagggtggttaggacagc

SEQ ID NO: 174 - DNA, 58 bp, synthetic construct
  source 1..58: mol_type = other DNA
  modified_base order(26,32,42): mod_base = OTHER; note = an unnatural base
gtccgttcacggcaaacgcactttantggtgngggtgggctngtcttcgtgaacggac

SEQ ID NO: 175 - DNA, 58 bp, synthetic construct
  source 1..58: mol_type = other DNA
  modified_base order(16,28,33): mod_base = OTHER; note = an unnatural base
gtcctttcacgtagcnggtccgggttantgggngggtggcttggggccgtgaaaggac

SEQ ID NO: 176 - DNA, 59 bp, synthetic construct
  source 1..59: mol_type = other DNA
  modified_base order(15,23,34): mod_base = OTHER; note = an unnatural base
gcgtgcgtgaagttngggtgggnatgtgatgggnggtagatacgcaacgccgcgtagcg

SEQ ID NO: 177 - DNA, 57 bp, synthetic construct; identical to SEQ ID NO: 142
  source 1..57: mol_type = other DNA
  modified_base order(16,22): mod_base = OTHER; note = an unnatural base

SEQ ID NO: 178 - DNA, 52 bp, synthetic construct
  source 1..52: mol_type = other DNA
  modified_base order(10,16,28): mod_base = OTHER; note = an unnatural base
gcacgctttnacttantggctgggtggnctgggtaaagcgtgccgcgtagcg

SEQ ID NO: 179 - DNA, 40 bp, synthetic construct
  source 1..40: mol_type = other DNA
gtgacgtaggttggtgtggttggggcgtcaccgcgtagcg

SEQ ID NO: 180 - DNA, 47 bp, synthetic construct; identical to SEQ ID NO: 26
  source 1..47: mol_type = other DNA
  modified_base order(24,33): mod_base = OTHER; note = an unnatural base

SEQ ID NO: 181 - DNA, 49 bp, synthetic construct; identical to SEQ ID NO: 18
  source 1..49: mol_type = other DNA
  modified_base order(18,29,40): mod_base = OTHER; note = an unnatural base

SEQ ID NO: 182 - DNA, 44 bp, synthetic construct; identical to SEQ ID NO: 4
  source 1..44: mol_type = other DNA
  modified_base order(10,22,33): mod_base = OTHER; note = an unnatural base

SEQ ID NO: 183 - DNA, 31 bp, synthetic construct; identical to SEQ ID NO: 30
  source 1..31: mol_type = other DNA
  modified_base order(15,21): mod_base = OTHER; note = an unnatural base

SEQ ID NO: 184 - DNA, 51 bp, synthetic construct
  source 1..51: mol_type = other DNA
  modified_base order(5,17,29): mod_base = OTHER; note = an unnatural base
tccgnctgggaacaagnggcgggagggangggtgtgggtgcgacaagcgga

SEQ ID NO: 185 - DNA, 42 bp, synthetic construct; identical to SEQ ID NO: 41
  source 1..42: mol_type = other DNA
  modified_base order(11,19): mod_base = OTHER; note = an unnatural base

SEQ ID NO: 186 - DNA, 40 bp, synthetic construct
  source 1..40: mol_type = other DNA
  modified_base order(14,24): mod_base = OTHER; note = an unnatural base
ggagacgtaacgcntatcaaatcnaaacagcttagggtcc

SEQ ID NO: 187 - DNA, 28 bp, synthetic construct
  source 1..28: mol_type = other DNA
  modified_base order(3,24): mod_base = OTHER; note = an unnatural base
gangagcaccgaaggtctcaacgntgga

SEQ ID NO: 188 - DNA, 36 bp, synthetic construct
  source 1..36: mol_type = other DNA
  modified_base order(22,33): mod_base = OTHER; note = an unnatural base
cgggtccgcgaagcggtaggtntgggctaggcngct

SEQ ID NO: 189 - DNA, 36 bp, synthetic construct; identical to SEQ ID NO: 63
  source 1..36: mol_type = other DNA
  modified_base order(15,28): mod_base = OTHER; note = an unnatural base

SEQ ID NO: 190 - DNA, 30 bp, synthetic construct
  source 1..30: mol_type = other DNA
  modified_base order(7,13): mod_base = OTHER; note = an unnatural base
tgtggtngttttnttgggggggtggttaag

SEQ ID NO: 191 - DNA, 49 bp, synthetic construct
  source 1..49: mol_type = other DNA
  modified_base order(25,34): mod_base = OTHER; note = an unnatural base
gcggtaagccgcgtccgaaggggcntgcggcgancccgaatgggtccgc

SEQ ID NO: 192 - DNA, 41 bp, synthetic construct
  source 1..41: mol_type = other DNA
  modified_base order(21,30): mod_base = OTHER; note = an unnatural base
taagccgcgtccgaaggggcntgcggcgancccgaatgggt

SEQ ID NO: 193 - DNA, 52 bp, synthetic construct
  source 1..52: mol_type = other DNA
  modified_base order(22,33): mod_base = OTHER; note = an unnatural base
ctccttcagcgccaccgtatgnacgctcacagnagttgccgagctgaaggag

SEQ ID NO: 194 - DNA, 32 bp, synthetic construct
  source 1..32: mol_type = other DNA
  modified_base order(12,23): mod_base = OTHER; note = an unnatural base
gccaccgtatgnacgctcacagnagttgccga

SEQ ID NO: 195 - DNA, 36 bp, synthetic construct
  source 1..36: mol_type = other DNA
  modified_base 27: mod_base = OTHER; note = an unnatural base
ggcgccaggggtgtttgtgccgtgagntgtggcgcc

SEQ ID NO: 196 - DNA, 22 bp, synthetic construct
  source 1..22: mol_type = other DNA
  modified_base 20: mod_base = OTHER; note = an unnatural base
ggggtgtttgtgccgtgagntg

SEQ ID NO: 197 - DNA, 19 bp, synthetic construct
  source 1..19: mol_type = other DNA
  modified_base order(9,15): mod_base = OTHER; note = an unnatural base
actggtgtnctcggnatgg

SEQ ID NO: 198 - DNA, 42 bp, synthetic construct
  source 1..42: mol_type = other DNA
  modified_base order(14,27): mod_base = OTHER; note = an unnatural base
ggtccggcccgtantcagacgtatacncatcagggccggacc

SEQ ID NO: 199 - DNA, 22 bp, synthetic construct
  source 1..22: mol_type = other DNA
  modified_base order(4,17): mod_base = OTHER; note = an unnatural base
gtantcagacgtatacncatca

SEQ ID NO: 200 - DNA, 44 bp, synthetic construct
  source 1..44: mol_type = other DNA
  modified_base 13: mod_base = OTHER; note = an unnatural base
ggctggtccgcgnccaacctccaccaatcaaagccggaccagcc

SEQ ID NO: 201 - DNA, 24 bp, synthetic construct
  source 1..24: mol_type = other DNA
  modified_base 3: mod_base = OTHER; note = an unnatural base
cgnccaacctccaccaatcaaagc

SEQ ID NO: 202 - DNA, 30 bp, synthetic construct
  source 1..30: mol_type = other DNA
  modified_base order(5,13): mod_base = OTHER; note = an unnatural base
tctancctggccntgtggtactgtaacggc

SEQ ID NO: 203 - DNA, 48 bp, synthetic construct
  source 1..48: mol_type = other DNA
  modified_base order(18,28): mod_base = OTHER; note = unnatural base
cggcggagacgtaacgcntatcaaatcnaaacagcttagggtccgccg

SEQ ID NO: 204 - DNA, 34 bp, synthetic construct
  source 1..34: mol_type = other DNA
  modified_base order(11,21): mod_base = OTHER; note = an unnatural base
gacgtaacgcntatcaaatcnaaacagcttaggg

SEQ ID NO: 205 - DNA, 25 bp, synthetic construct
  source 1..25: mol_type = other DNA
  modified_base order(3,24): mod_base = OTHER; note = an unnatural base
gangagyaccgaaggtctcrryrny

SEQ ID NO: 206 - DNA, 30 bp, synthetic construct
  source 1..30: mol_type = other DNA
  modified_base order(3,15,26): mod_base = OTHER; note = an unnatural base
gangagyacctaacnggtctcrryrnygga

SEQ ID NO: 207 - DNA, 36 bp, synthetic construct
  source 1..36: mol_type = other DNA
  modified_base order(22,33): mod_base = OTHER; note = an unnatural base
cgggtccgcgaagcggtaggtnygggctaggcngyy

SEQ ID NO: 208 - DNA, 37 bp, synthetic construct
  source 1..37: mol_type = other DNA
  modified_base order(12,23,34): mod_base = OTHER; note = an unnatural base
cgggtcatttantaatgtaggtnygggctaggcngyy

SEQ ID NO: 209 - DNA, 41 bp, synthetic construct
  source 1..41: mol_type = other DNA
  modified_base order(21,30): mod_base = OTHER; note = an unnatural base
taaactgcgtccgaaggggcntgcagtgancccgaatgggt

SEQ ID NO: 210 - DNA, 19 bp, synthetic construct
  source 1..19: mol_type = other DNA
  modified_base order(11,17): mod_base = OTHER; note = an unnatural base
rctggtgynctcggnatgr

SEQ ID NO: 211 - DNA, 19 bp, synthetic construct
  source 1..19: mol_type = other DNA
  modified_base order(11,17): mod_base = OTHER; note = an unnatural base
rctggtgynctcggnatgr

SEQ ID NO: 212 - DNA, 54 bp, synthetic construct; identical to SEQ ID NO: 145
  source 1..54: mol_type = other DNA
  modified_base 37: mod_base = OTHER; note = an unnatural base

SEQ ID NO: 213 - DNA, 36 bp, synthetic construct
  source 1..36: mol_type = other DNA
  modified_base 28: mod_base = OTHER; note = an unnatural base
ccgtcataattgttattttgatccttgnagtgggga

SEQ ID NO: 214 - skipped